European Patent Application EP 4 382 608 A1, published June 12, 2024. Title: 新規フラビン依存性乳酸デヒドロゲナーゼ及び乳酸デヒドロゲナーゼの安定性を向上させる方法. Applicant: KIKKOMAN CORPORATION. Application JP. The sequence listing filed with the application follows.

SEQUENCE LISTING (27 sequences)

SEQ ID NO: 1 - protein, 578 aa, enzyme
MLLRSLNSSARCVKQTTRTKVRYLSHVSGASMAKPTLKNNSRESNKSRNYLIAAVTALAVSTSIGVAVHVKDPLYNDATGSDSPRSISVDEFVKHNSQNDCWIAINGKVYDFTDFIPNHPGGVPPLVNHAGYDGTKLYEKLHPKGTIEKFLPKDKFLGVLDGEAPKLEADYLVDDDEQERLDYLNNLPPLSSIQNVYDFEYLAKKILPKDAWAYYSCGADDEITMRENHYAYQRVYFRPRICVDVKEVDTSYEMLGTKTSVPFYVSATALAKLGHPDGECSIARGAGKEGVVQMISTLSSMSLDEIAAARIPGATQWFQLYINEDRNVAKGLVKHAEDLGMKAIFITVDAPSLGNREKDKRLKFVNDTDVDLGDSADRNSGASKALSSFIDASVSWNDVKAVKSWTKLPVLVKGVQTVEDVIEAYDAGCQGVVLSNHGGRQLDTAPPPIELLAETVPTLKRLGKLRPDFEILIDGGVKRGTDILKAVAIGGQDVRVSVGMGRPFLYANSCYGEAGVRKLIQNLKDELEMDMRLLGVTKMDQLSSKHVDTKRLIGRDAINYLYDNVYSPIETVKFNNED

SEQ ID NO: 2 - protein, 506 aa, enzyme
MNKQKISPAEVAKHNKPDDCWVVINGYVYDLTRFLPNHPGGQDVIKFNAGKDVTAIFEPLHAPNVIDKYIAPEKKLGPLQGSMPPELVCPPYAPGETKEDIARKEQLKSLLPPLDNIINLYDFEYLASQTLTKQAWAYYSSGANDEVTHRENHNAYHRIFFKPKILVDVRKVDISTDMLGSHVDVPFYVSATALCKLGNPLEGEKDVARGCGQGVTKVPQMISTLASCSPEEIIEAAPSDKQIQWYQLYVNSDRKITDDLVKNVEKLGVKALFVTVDAPSLGQREKDMKLKFSNTKAGPKAMKKTNVEESQGASRALSKFIDPSLTWKDIEELKKKTKLPIVIKGVQRTEDVIKAAEIGVSGVVLSNHGGRQLDFSRAPIEVLAETMPILEQRNLKDKLEVFVDGGVRRGTDVLKALCLGAKGVGLGRPFLYANSCYGRNGVEKAIEILRDEIEMSMRLLGVTSIAELKPDLLDLSTLKARTVGVPNDVLYNEVYEGPTLTEFEDA

SEQ ID NO: 3 - protein, 502 aa, enzyme
MATGSDSPRSISVDEFVKHNSQNDCWIAINGKVYDFTDFIPNHPGGVPPLVNHAGYDGTKLYEKLHPKGTIEKFLPKDKFLGVLDGEAPKLEADYLVDDDEQERLDYLNNLPPLSSIQNVYDFEYLAKKILPKDAWAYYSCGADDEITMRENHYAYQRVYFRPRICVDVKEVDTSYEMLGTKTSVPFYVSATALAKLGHPDGECSIARGAGKEGVVQMISTLSSMSLDEIAAARIPGATQWFQLYINEDRNVAKGLVKHAEDLGMKAIFITVDAPSLGNREKDKRLKFVNDTDVDLGDSADRNSGASKALSSFIDASVSWNDVKAVKSWTKLPVLVKGVQTVEDVIEAYDAGCQGVVLSNHGGRQLDTAPPPIELLAETVPTLKRLGKLRPDFEILIDGGVKRGTDILKAVAIGGQDVRVSVGMGRPFLYANSCYGEAGVRKLIQNLKDELEMDMRLLGVTKMDQLSSKHVDTKRLIGRDAINYLYDNVYSPIETVKFNNED

SEQ ID NO: 4 - DNA, 1509 bp, enzyme
  source 1..1509: mol_type = other DNA
atggctactgggtcagatagtcctagaagcattagcgttgacgaattcgttaaacacaacagccagaatgattgttggattgccattaatggaaaagtttatgatttcacggatttcattcctaaccacccagggggtgtcccacccctggtgaatcacgccggttacgacggtacgaaactgtatgaaaaactgcatcctaaaggtaccattgaaaaatttttaccgaaagataaatttcttggcgtgttagacggcgaggctccgaagctggaggcggattacctggttgacgacgacgaacaggaaagactggactacttgaacaatttgccgcctttatccagtattcagaatgtctacgacttcgagtatttggcaaaaaagattctgcctaaggatgcttgggcctactacagctgcggtgcagatgacgagataacgatgcgcgaaaaccattatgcgtatcaacgcgtttacttccgtccgcgcatttgcgttgatgtgaaggaagttgatactagctatgaaatgctgggtactaaaaccagcgtgccgttttatgttagtgccaccgcattggcgaaactgggtcatcccgatggtgagtgctcaattgcacgtggcgctggtaaggaaggtgtcgttcagatgatttcaactctgtcatcaatgagtctggatgaaatagcggcggcacggattccaggggcgacccagtggtttcagctgtatattaatgaggatcgtaatgtcgctaagggtctggttaaacatgcagaagacctgggtatgaaggcaatttttataaccgtggacgcaccgtccttaggcaatcgtgagaaggataagcgtctgaaatttgttaacgacacggatgtagatctgggggactcagccgaccgtaattcgggagcgtccaaggctctgagttcgtttatagatgcaagtgtttcttggaacgatgtgaaagccgtgaagtcgtggaccaaattacccgtgctggttaaaggagttcagaccgtggaagatgtaatagaagcctatgatgcaggttgtcagggggtcgtactgtctaaccatggagggcgccaactggacactgccccaccaccgatcgaacttctggcagagacggtgccgacattgaaacgtttaggcaaattacgcccggattttgaaatcttaatcgatggcggcgtgaaacgtgggacagacatattaaaagccgtggcgatcggcggccaagatgtaagagtatctgtaggcatgggacgcccatttttatatgctaactcttgttatggagaggcgggagtccggaaattgatccaaaatttgaaagatgagcttgaaatggatatgcgccttcttggcgtcacaaaaatggatcaactttcttctaaacatgtagatacaaaacggcttatcggacgggatgctatcaactatctttatgataatgtatattcccctatcgaaacagtcaaatttaataatgaagattaa

SEQ ID NO: 5 - protein, 500 aa, enzyme
MGSDSPRSISVDEFVKHNRPDDCWVAIRGQVYDMTEFLPHHPGGQSPIIRYSGHDATELFEQLHPKGTIEKHLPKEKHLGQLDGPAPTLEADYLVDDDEQERLDYLNNLPPLSSIQNVYDFEYLAKKILPKDAWAYYSCGADDEITMRENHYAFQRVYFRPRICVDVKEVDTSYEMLGTKTSVPFYVSATALAKLGHPDGECSIARGAGKEGVVQMISTLSSMSLDEIAAARIPGATQWFQLYINEDRNVAKGLVKHAEDLGMKAIFITVDAPSLGNREKDKRLKFVNDTDVDLGDSADRNSGASKALSSFIDASVSWNDVKAVKSWTKLPVLVKGVQTVEDVIEAFDAGCQGVVLSNHGGRQLDTAPPPIELLAETVPTLKRLGKLRPDFEILIDGGVKRGTDILKAVAIGGQDVRVSVGMGRPLLYANSCYGEAGVRKLIQNLKDELEMDMRLLGVTKMDQLSSKHVDTKRLIGRDAINYLYDNVYSPIETVKFNNED

SEQ ID NO: 6 - DNA, 1503 bp, enzyme
  source 1..1503: mol_type = other DNA
atggggtcagatagtcctagaagcattagcgttgacgaattcgttaaacacaatcgtcccgatgactgctgggttgcgatacggggtcaggtttatgatatgacggagttcctgccgcaccatcctggcggtcagagccctattatacgttattcaggccacgatgcaacggagcttttcgaacaattgcatcctaagggtacaattgaaaagcatttaccgaaagagaagcatttgggccaactggatggtccggcccctaccctggaagcggattacctggttgacgacgacgaacaggaaagactggactacttgaacaatttgccgcctttatccagtattcagaatgtctacgacttcgagtatttggcaaaaaagattctgcctaaggatgcttgggcctactacagctgcggtgcagatgacgagataacgatgcgcgaaaaccattatgcgtttcaacgcgtttacttccgtccgcgcatttgcgttgatgtgaaggaagttgatactagctatgaaatgctgggtactaaaaccagcgtgccgttttatgttagtgccaccgcattggcgaaactgggtcatcccgatggtgagtgctcaattgcacgtggcgctggtaaggaaggtgtcgttcagatgatttcaactctgtcatcaatgagtctggatgaaatagcggcggcacggattccaggggcgacccagtggtttcagctgtatattaatgaggatcgtaatgtcgctaagggtctggttaaacatgcagaagacctgggtatgaaggcaatttttataaccgtggacgcaccgtccttaggcaatcgtgagaaggataagcgtctgaaatttgttaacgacacggatgtagatctgggggactcagccgaccgtaattcgggagcgtccaaggctctgagttcgtttatagatgcaagtgtttcttggaacgatgtgaaagccgtgaagtcgtggaccaaattacccgtgctggttaaaggagttcagaccgtggaagatgtaatagaagcctttgatgcaggttgtcagggggtcgtactgtctaaccatggagggcgccaactggacactgccccaccaccgatcgaacttctggcagagacggtgccgacattgaaacgtttaggcaaattacgcccggattttgaaatcttaatcgatggcggcgtgaaacgtgggacagacatattaaaagccgtggcgatcggcggccaagatgtaagagtatctgtaggcatgggacgcccattattatatgctaactcttgttatggagaggcgggagtccggaaattgatccaaaatttgaaagatgagcttgaaatggatatgcgccttcttggcgtcacaaaaatggatcaactttcttctaaacatgtagatacaaaacggcttatcggacgggatgctatcaactatctttatgataatgtatattcccctatcgaaacagtcaaatttaataatgaagattaa

SEQ ID NO: 7 - DNA, 39 bp, synthetic construct
  misc_feature 1..39: note = none
  source 1..39: mol_type = other DNA
cccctggtgaatcactgcggttacgacggtacgaaactg

SEQ ID NO: 8 - DNA, 28 bp, synthetic construct
  misc_feature 1..28: note = none
  source 1..28: mol_type = other DNA
gtgattcaccaggggtgggacaccccct

SEQ ID NO: 9 - DNA, 28 bp, synthetic construct
  misc_feature 1..28: note = none
  source 1..28: mol_type = other DNA
cgttattgcggccacgatgcaacggagc

SEQ ID NO: 10 - DNA, 28 bp, synthetic construct
  misc_feature 1..28: note = none
  source 1..28: mol_type = other DNA
gtggccgcaataacgtataatagggctc

SEQ ID NO: 11 - DNA, 30 bp, synthetic construct
  misc_feature 1..30: note = none
  source 1..30: mol_type = other DNA
catgaatcctgtttcctgtgtgaaattgtt

SEQ ID NO: 12 - DNA, 30 bp, synthetic construct
  misc_feature 1..30: note = none
  source 1..30: mol_type = other DNA
ccgaaagataaatttcttggcgtgttagac

SEQ ID NO: 13 - DNA, 30 bp, synthetic construct
  misc_feature 1..30: note = none
  source 1..30: mol_type = other DNA
ttagacggcgaggctccgaagctggaggcg

SEQ ID NO: 14 - DNA, 30 bp, synthetic construct
  misc_feature 1..30: note = none
  source 1..30: mol_type = other DNA
gaggcggattacctggttgacgacgacgaa

SEQ ID NO: 15 - DNA, 30 bp, synthetic construct
  misc_feature 1..30: note = none
  source 1..30: mol_type = other DNA
actgggtcagatagtcctagaagcattagc

SEQ ID NO: 16 - DNA, 30 bp, synthetic construct
  misc_feature 1..30: note = none
  source 1..30: mol_type = other DNA
gggtcagatagtcctagaagcattagcgtt

SEQ ID NO: 17 - DNA, 30 bp, synthetic construct
  misc_feature 1..30: note = none
  source 1..30: mol_type = other DNA
tcagatagtcctcgtagcattagcgttgac

SEQ ID NO: 18 - DNA, 30 bp, synthetic construct
  misc_feature 1..30: note = none
  source 1..30: mol_type = other DNA
gatagtcctcgtagcattagcgttgacgaa

SEQ ID NO: 19 - DNA, 30 bp, synthetic construct
  misc_feature 1..30: note = none
  source 1..30: mol_type = other DNA
agtcctcgtagcattagcgttgacgaattc

SEQ ID NO: 20 - DNA, 30 bp, synthetic construct
  misc_feature 1..30: note = none
  source 1..30: mol_type = other DNA
cctcgtagcattagcgttgacgaattcgtt

SEQ ID NO: 21 - DNA, 30 bp, synthetic construct
  misc_feature 1..30: note = none
  source 1..30: mol_type = other DNA
atgggacgcccattattatatgctaactct

SEQ ID NO: 22 - DNA, 30 bp, synthetic construct
  misc_feature 1..30: note = none
  source 1..30: mol_type = other DNA
tgggcgtcccatgcctacagatactcttac

SEQ ID NO: 23 - DNA, 30 bp, synthetic construct
  misc_feature 1..30: note = none
  source 1..30: mol_type = other DNA
cgcataatggttttcgcgcatcgttatctc

SEQ ID NO: 24 - DNA, 30 bp, synthetic construct
  misc_feature 1..30: note = none
  source 1..30: mol_type = other DNA
aaccattatgcgtttcaacgcgtttacttc

SEQ ID NO: 25 - DNA, 30 bp, synthetic construct
  misc_feature 1..30: note = none
  source 1..30: mol_type = other DNA
ggcttctattacatcttccacggtctgaac

SEQ ID NO: 26 - DNA, 30 bp, synthetic construct
  misc_feature 1..30: note = none
  source 1..30: mol_type = other DNA
gtaatagaagcctttgatgcaggttgtcag

SEQ ID NO: 27 - DNA, 30 bp, synthetic construct
  misc_feature 1..30: note = none
  source 1..30: mol_type = other DNA
aatttgccgcctttatccagtattcagaat